European Patent Application EP 4 324 844 A1, published February 21, 2024. Title: Use Novel Light Sensitive Channel Protein VR1.0 in Preparation of Retinal Photoreceptor Cell Degenerative Disease Drug. Applicant: Zhongmou Medical Technology (Wuhan) Co., Ltd. The sequence listing filed with the application follows.

SEQUENCE LISTING (2 sequences)

SEQ ID NO: 1 - protein, 341 aa, Artificial Sequence
  VR1.0
MRPQILLLLALLTLGLANGTEGPNFYVPFSNKTGVVRSMGFQLNPEYLNETILLDDCTPIYLNVGPLWEQKVARGTQWFGVILSLAFLIYYIWITYKATCGWEELYVCTIEFCKIVIELYFEFSPPAMIYQTNGEVTPWLRYAEWLLTCPVICIHLSNITGLNDDYSGRTMSLITSDLGGICMAVTSALSKGWLKWLFFVIGCCYGASTFYHAALIYIESYYTMPHGVCKNMVLAMAAVFFTSWFMFPGLFLAGPEGTNALSWAGSTIGHTVADLLSKNAWGMIGHFLRLEIHKHIIIHGDVRRPITVNTLGREVTVSCFVDKEEEDEDERISTKTYANRA

SEQ ID NO: 2 - DNA, 1023 bp, Artificial Sequence
  Encoding gene sequence of VR1.0
atgcgaccccaaatactcctcttgctggctttgttgacccttggactggctaacggaacagaaggtcccaacttctacgttcctttcagcaataagacaggcgtagtcagatccatgggcttccagctcaatccggaatacctgaacgaaacaattttgctggacgactgtacgccaatctatctgaacgtcggtcccctgtgggagcaaaaggttgcccgaggtacgcaatggtttggtgttatcctctcgttggcgtttctcatctattatatatggataacatataaggcgacttgcggatgggaagaactgtacgtgtgtacgatcgaattttgtaaaattgtaattgaactctacttcgagttttcgcctccggcgatgatatatcagaccaacggagaggtaacgccctggttgcgatatgctgaatggctcttgacctgcccagtcatttgcatacatttgagtaacattacaggactcaatgacgactattcgggccgaactatgtccctgatcacatccgacctgggaggcatctgcatggccgttacttccgccttgagtaaaggctggttgaagtggctctttttcgtgatcggctgttgttacggtgctagtacgttttatcatgcggcgctcatatatatagaaagttactacactatgcctcacggtgtttgtaaaaacatggtattggcgatggcagcggtattttttacaagttggttcatgtttcccggtttgttcctggcaggccctgaaggaaccaatgcactgtcgtgggcgggctcgactatcggtcataccgtggcagatttgctctccaaaaacgcctggggtatgattggtcacttcctccgactggagatacacaaacatataattattcatggtgatgttcgtcgcccgataacggttaataccttgggacgagaagtcacggtgtcgtgttttgtcgataaagaagaggaggatgaagacgaacgtatcagcactaagacctacgcgaaccgggca